European Patent Application EP 4 299 756 A1, published January 3, 2024. Title: Method of Production of Antibody-Lysosomal Enzyme Fusion Protein. Applicant: JCR Pharmaceuticals Co., Ltd. The sequence listing filed with the application follows.

SEQUENCE LISTING (42 sequences)

SEQ ID NO: 1 - protein, 5 aa, Artificial Sequence
  Amino acid sequence of an exemplified linker 1
GGGGS

SEQ ID NO: 2 - protein, 6 aa, Artificial Sequence
  Amino acid sequence of an exemplified linker 2
GGGGGS

SEQ ID NO: 3 - protein, 5 aa, Artificial Sequence
  Amino acid sequence of an exemplified linker 3
SGGGG

SEQ ID NO: 4 - protein, 15 aa, Artificial Sequence
  Amino acid sequence of an exemplified linker 4
GGGGSGGGGSGGGGS

SEQ ID NO: 5 - protein, 760 aa, Homo sapiens
MMDQARSAFSNLFGGEPLSYTRFSLARQVDGDNSHVEMKLAVDEEENADNNTKANVTKPKRCSGSICYGTIAVIVFFLIGFMIGYLGYCKGVEPKTECERLAGTESPVREEPGEDFPAARRLYWDDLKRKLSEKLDSTDFTGTIKLLNENSYVPREAGSQKDENLALYVENQFREFKLSKVWRDQHFVKIQVKDSAQNSVIIVDKNGRLVYLVENPGGYVAYSKAATVTGKLVHANFGTKKDFEDLYTPVNGSIVIVRAGKITFAEKVANAESLNAIGVLIYMDQTKFPIVNAELSFFGHAHLGTGDPYTPGFPSFNHTQFPPSRSSGLPNIPVQTISRAAAEKLFGNMEGDCPSDWKTDSTCRMVTSESKNVKLTVSNVLKEIKILNIFGVIKGFVEPDHYVVVGAQRDAWGPGAAKSGVGTALLLKLAQMFSDMVLKDGFQPSRSIIFASWSAGDFGSVGATEWLEGYLSSLHLKAFTYINLDKAVLGTSNFKVSASPLLYTLIEKTMQNVKHPVTGQFLYQDSNWASKVEKLTLDNAAFPFLAYSGIPAVSFCFCEDTDYPYLGTTMDTYKELIERIPELNKVARAAAEVAGQFVIKLTHDVELNLDYERYNSQLLSFVRDLNQYRADIKEMGLSLQWLYSARGDFFRATSRLTTDFGNAEKTDRFVMKKLNDRVMRVEYHFLSPYVSPKESPFRHVFWGSGSHTLPALLENLKLRKQNNGAFNETLFRNQLALATWTIQGAANALSGDVWDIDNEF

SEQ ID NO: 6 - protein, 628 aa, Homo sapiens
AEAPHLVHVDAARALWPLRRFWRSTGFCPPLPHSQADQYVLSWDQQLNLAYVGAVPHRGIKQVRTHWLLELVTTRGSTGRGLSYNFTHLDGYLDLLRENQLLPGFELMGSASGHFTDFEDKQQVFEWKDLVSSLARRYIGRYGLAHVSKWNFETWNEPDHHDFDNVSMTMQGFLNYYDACSEGLRAASPALRLGGPGDSFHTPPRSPLSWGLLRHCHDGTNFFTGEAGVRLDYISLHRKGARSSISILEQEKVVAQQIRQLFPKFADTPIYNDEADPLVGWSLPQPWRADVTYAAMVVKVIAQHQNLLLANTTSAFPYALLSNDNAFLSYHPHPFAQRTLTARFQVNNTRPPHVQLLRKPVLTAMGLLALLDEEQLWAEVSQAGTVLDSNHTVGVLASAHRPQGPADAWRAAVLIYASDDTRAHPNRSVAVTLRLRGVPPGPGLVYVTRYLDNGLCSPDGEWRRLGRPVFPTAEQFRRMRAAEDPVAAAPRPLPAGGRLTLRPALRLPSLLLVHVCARPEKPPGQVTRLRALPLTQGQLVLVWSDEHVGSKCLWTYEIQFSQDGKAYTPVSRKPSTFNLFVFSPDTGAVSGSYRVRALDYWARPGPFSDPVPYLEVPVPRGPPSPGNP

SEQ ID NO: 7 - protein, 626 aa, Homo sapiens
APHLVHVDAARALWPLRRFWRSTGFCPPLPHSQADQYVLSWDQQLNLAYVGAVPHRGIKQVRTHWLLELVTTRGSTGRGLSYNFTHLDGYLDLLRENQLLPGFELMGSASGHFTDFEDKQQVFEWKDLVSSLARRYIGRYGLAHVSKWNFETWNEPDHHDFDNVSMTMQGFLNYYDACSEGLRAASPALRLGGPGDSFHTPPRSPLSWGLLRHCHDGTNFFTGEAGVRLDYISLHRKGARSSISILEQEKVVAQQIRQLFPKFADTPIYNDEADPLVGWSLPQPWRADVTYAAMVVKVIAQHQNLLLANTTSAFPYALLSNDNAFLSYHPHPFAQRTLTARFQVNNTRPPHVQLLRKPVLTAMGLLALLDEEQLWAEVSQAGTVLDSNHTVGVLASAHRPQGPADAWRAAVLIYASDDTRAHPNRSVAVTLRLRGVPPGPGLVYVTRYLDNGLCSPDGEWRRLGRPVFPTAEQFRRMRAAEDPVAAAPRPLPAGGRLTLRPALRLPSLLLVHVCARPEKPPGQVTRLRALPLTQGQLVLVWSDEHVGSKCLWTYEIQFSQDGKAYTPVSRKPSTFNLFVFSPDTGAVSGSYRVRALDYWARPGPFSDPVPYLEVPVPRGPPSPGNP

SEQ ID NO: 8 - protein, 11 aa, Artificial Sequence
  Amino acid sequence 1 of CDR 1 in the light chain of anti-hTfR antibody
QSLVHSNGNTY

SEQ ID NO: 9 - protein, 16 aa, Artificial Sequence
  Amino acid sequence 2 of CDR 1 in the light chain of  anti-hTfR antibody
RSSQSLVHSNGNTYLH

SEQ ID NO: 10 - protein, 6 aa, Artificial Sequence
  Amino acid sequence 1 of CDR 2 in the light chain of anti-hTfR antibody
KVSNRF

SEQ ID NO: 11 - protein, 7 aa, Artificial Sequence
  Amino acid sequence 2 of CDR 2 in the light chain of anti-hTfR antibody
KVSNRFS

SEQ ID NO: 12 - protein, 9 aa, Artificial Sequence
  Amino acid sequence of CDR 3 in the light chain of anti-hTfR antibody
SQSTHVPWT

SEQ ID NO: 13 - protein, 8 aa, Artificial Sequence
  Amino acid sequence 1 of CDR1 in the heavy chain of anti-h s   q antibody
GYSFMNYW

SEQ ID NO: 14 - protein, 10 aa, Artificial Sequence
  Amino acid sequence 2 of CDR1 in the heavy chain of anti-h s   q antibody
GYSFMNYWLG

SEQ ID NO: 15 - protein, 8 aa, Artificial Sequence
  Amino acid sequence 1 of CDR 2 in the heavy chain of anti-hTfR antibody
IYPGGDYP

SEQ ID NO: 16 - protein, 17 aa, Artificial Sequence
  Amino acid sequence 2 of CDR 2 in the heavy chain of anti-hTfR antibody
DIYPGGDYPTYSEKFKV

SEQ ID NO: 17 - protein, 9 aa, Artificial Sequence
  Amino acid sequence 1 of CDR 3 in the heavy chain of anti-hTfR antibody
SGNYDEVAY

SEQ ID NO: 18 - protein, 11 aa, Artificial Sequence
  Amino acid sequence 2 of CDR 3 in the heavy chain of anti-hTfR antibody
ARSGNYDEVAY

SEQ ID NO: 19 - protein, 30 aa, Artificial Sequence
  Amino acid sequence of framework region 3 in the heavy chain of anti-h s   q antibody
QVTISADKSISTAYLQLSSLKASDTAMYYC

SEQ ID NO: 20 - protein, 112 aa, Artificial Sequence
  Amino acid sequence of the variable region of the light chain ofanti-hTfR antibody
DIVMTQTPLSLSVTPGQPASISCRSSQSLVHSNGNTYLHWYLQKPGQSPQLLIYKVSNRFSGVPDRFSGSGSGTDFTLKISRVEAEDVGVYYCSQSTHVPWTFGQGTKVEIK

SEQ ID NO: 21 - protein, 118 aa, Artificial Sequence
  Amino acid sequence of the variable region of the heavy chain of anti-h s   q antibody
EVQLVQSGAEVKKPGESLKISCKGSGYSFMNYWLGWVRQMPGKGLEWMGDIYPGGDYPTYSEKFKVQVTISADKSISTAYLQLSSLKASDTAMYYCARSGNYDEVAYWGQGTLVTVSS

SEQ ID NO: 22 - protein, 219 aa, Artificial Sequence
  Amino acid sequence of the light chain of anti-hTfR antibody
DIVMTQTPLSLSVTPGQPASISCRSSQSLVHSNGNTYLHWYLQKPGQSPQLLIYKVSNRFSGVPDRFSGSGSGTDFTLKISRVEAEDVGVYYCSQSTHVPWTFGQGTKVEIKRTVAAPSVFIFPPSDEQLKSGTASVVCLLNNFYPREAKVQWKVDNALQSGNSQESVTEQDSKDSTYSLSSTLTLSKADYEKHKVYACEVTHQGLSSPVTKSFNRGEC

SEQ ID NO: 23 - protein, 226 aa, Artificial Sequence
  Amino acid sequence of Fab heavy chain of anti-h s   q antibody
EVQLVQSGAEVKKPGESLKISCKGSGYSFMNYWLGWVRQMPGKGLEWMGDIYPGGDYPTYSEKFKVQVTISADKSISTAYLQLSSLKASDTAMYYCARSGNYDEVAYWGQGTLVTVSSASTKGPSVFPLAPSSKSTSGGTAALGCLVKDYFPEPVTVSWNSGALTSGVHTFPAVLQSSGLYSLSSVVTVPSSSLGTQTYICNVNHKPSNTKVDKKVEPKSCDKTHT

SEQ ID NO: 24 - DNA, 20 bp, Artificial Sequence
  Primer Hyg-Sfi5', synthetic sequence
gaggccgcctcggcctctga

SEQ ID NO: 25 - DNA, 29 bp, Artificial Sequence
  Primer Hyg-BstX3', synthetic sequence
aaccatcgtgatgggtgctattcctttgc

SEQ ID NO: 26 - DNA, 740 bp, Artificial Sequence
  Nucleotide sequence encoding the amino acid sequence of the light chain ofanti-hTfR antibody, synthetic sequence
acgcgtgccgccaccatgggctggagctggattctgctgttcctcctgagcgtgacagcaggagtgcacagcgacatcgtgatgacccagactcccctgagcctgagcgtgacacctggccagcctgccagcatcagctgcagaagctctcagagcctggtgcacagcaacggcaacacctacctgcactggtatctgcagaagcccggccagagccctcagctgctgatctacaaggtgtccaacagattcagcggcgtgcccgacagattctccggcagcggctctggcaccgacttcaccctgaagatttccagagtggaagccgaggacgtgggcgtgtactactgcagccagagcacccacgtgccctggacattcggccagggcaccaaggtggaaatcaagagaaccgtggccgctcccagcgtgttcatcttcccacctagcgacgagcagctgaagtccggcacagcctctgtcgtgtgcctgctgaacaacttctacccccgcgaggccaaggtgcagtggaaggtggacaacgccctgcagagcggcaacagccaggaaagcgtgaccgagcaggactccaaggacagcacctacagcctgagcagcaccctgaccctgagcaaggccgactacgagaagcacaaggtgtacgcctgcgaagtgacccaccagggcctgtctagccccgtgaccaagagcttcaacagaggcgagtgctaagcggccgc

SEQ ID NO: 27 - protein, 869 aa, Artificial Sequence
  Amino acid sequence of fusion protein of the Fab heavy chain of anti-hTfR antibody and hIDUA
EVQLVQSGAEVKKPGESLKISCKGSGYSFMNYWLGWVRQMPGKGLEWMGDIYPGGDYPTYSEKFKVQVTISADKSISTAYLQLSSLKASDTAMYYCARSGNYDEVAYWGQGTLVTVSSASTKGPSVFPLAPSSKSTSGGTAALGCLVKDYFPEPVTVSWNSGALTSGVHTFPAVLQSSGLYSLSSVVTVPSSSLGTQTYICNVNHKPSNTKVDKKVEPKSCDKTHTGGGGSGGGGSGGGGSAEAPHLVHVDAARALWPLRRFWRSTGFCPPLPHSQADQYVLSWDQQLNLAYVGAVPHRGIKQVRTHWLLELVTTRGSTGRGLSYNFTHLDGYLDLLRENQLLPGFELMGSASGHFTDFEDKQQVFEWKDLVSSLARRYIGRYGLAHVSKWNFETWNEPDHHDFDNVSMTMQGFLNYYDACSEGLRAASPALRLGGPGDSFHTPPRSPLSWGLLRHCHDGTNFFTGEAGVRLDYISLHRKGARSSISILEQEKVVAQQIRQLFPKFADTPIYNDEADPLVGWSLPQPWRADVTYAAMVVKVIAQHQNLLLANTTSAFPYALLSNDNAFLSYHPHPFAQRTLTARFQVNNTRPPHVQLLRKPVLTAMGLLALLDEEQLWAEVSQAGTVLDSNHTVGVLASAHRPQGPADAWRAAVLIYASDDTRAHPNRSVAVTLRLRGVPPGPGLVYVTRYLDNGLCSPDGEWRRLGRPVFPTAEQFRRMRAAEDPVAAAPRPLPAGGRLTLRPALRLPSLLLVHVCARPEKPPGQVTRLRALPLTQGQLVLVWSDEHVGSKCLWTYEIQFSQDGKAYTPVSRKPSTFNLFVFSPDTGAVSGSYRVRALDYWARPGPFSDPVPYLEVPVPRGPPSPGNP

SEQ ID NO: 28 - DNA, 2688 bp, Artificial Sequence
  Nucleotide seuquence encoding the amino acid sequence of fusion protein of the Fab heavy chain of anti-hTfR antibody and hIDUA, synthetic sequence
acgcgtcgccaccatgggttggagcctcatcttgctcttccttgtcgctgttgctacgcgagtcggcagcgaggtgcaactagtgcagtctggagcagaggtgaaaaagcccggggagtctctgaagatttcctgtaagggttctggatacagctttatgaactactggctgggatgggtgcgccagatgcccgggaaaggcctggagtggatgggggacatctaccccggcggagactaccctacatacagcgagaagttcaaggtccaggtcaccatctcagccgacaagtccatcagcaccgcctacctgcagttgagcagcctgaaggcctcggacaccgccatgtattactgtgcgagatcaggcaattacgacgaagtggcctactggggccaaggaaccctggtcaccgtctcctcagctagcaccaagggcccatcggtcttccccctggcaccctcctccaagagcacctctgggggcacagcggccctgggctgcctggtcaaggactacttccccgaaccggtgacggtgtcgtggaactcaggcgccctgaccagcggcgtgcacaccttcccggctgtcctacagtcctcaggactctactccctcagcagcgtggtgaccgtgccctccagcagcttgggcacccagacctacatctgcaacgtgaatcacaagcccagcaacaccaaggtggacaagaaagttgagccgaagagctgtgataagacgcatacgggtggcggagggtctggaggtggcggatcaggcggaggtggatctgccgaggccccgcacctggtgcacgtggacgcggcccgcgcgctgtggcccctgcggcgcttctggaggagcacaggcttctgccccccgctgccacacagccaggctgaccagtacgtcctcagctgggaccagcagctcaacctcgcctatgtgggcgccgtccctcaccgcggcatcaagcaggtccggacccactggctgctggagcttgtcaccaccagggggtccactggacggggcctgagctacaacttcacccacctggacgggtacttggaccttctcagggagaaccagctcctcccagggtttgagctgatgggcagcgcctcgggccacttcactgactttgaggacaagcagcaggtgtttgagtggaaggacttggtctccagcctggccaggagatacatcggtaggtacggactggcgcatgtttccaagtggaacttcgagacgtggaatgagccagaccaccacgactttgacaacgtctccatgaccatgcaaggcttcctgaactactacgatgcctgctcggagggtctgcgcgccgccagccccgccctgcggctgggaggccccggcgactccttccacaccccaccgcgatccccgctgagctggggcctcctgcgccactgccacgacggtaccaacttcttcactggggaggcgggcgtgcggctggactacatctccctccacaggaagggtgcgcgcagctccatctccatcctggagcaggagaaggtcgtcgcgcagcagatccggcagctcttccccaagttcgcggacacccccatttacaacgacgaggcggacccgctggtgggctggtccctgccacagccgtggagggcggacgtgacctacgcggccatggtggtgaaggtcatcgcgcagcatcagaacctgctactggccaacaccacctccgccttcccctacgcgctcctgagcaacgacaatgccttcctgagctaccacccgcaccccttcgcgcagcgcacgctcaccgcgcgcttccaggtcaacaacacccgcccgccgcacgtgcagctgttgcgcaagccggtgctcacggccatggggctgctggcgctgctggatgaggagcagctctgggccgaagtgtcgcaggccgggaccgtcctggacagcaaccacacggtgggcgtcctggccagcgcccaccgcccccagggcccggccgacgcctggcgcgccgcggtgctgatctacgcgagcgacgacacccgcgcccaccccaaccgcagcgtcgcggtgaccctgcggctgcgcggggtgccccccggcccgggcctggtctacgtcacgcgctacctggacaacgggctctgcagccccgacggcgagtggcggcgcctgggccggcccgtcttccccacggcagagcagttccggcgcatgcgcgcggctgaggacccggtggccgcggcgccccgccccttacccgccggtggccgcctgaccctgcgccccgcgctgcggctgccgtcgcttttgctggtgcacgtgtgtgcgcgccccgagaagccgcccgggcaggtcacgcggctccgcgccctgcccctgacccaagggcagctggttctggtctggtcggatgaacacgtgggctccaagtgcctgtggacatacgagatccagttctctcaggacggtaaggcgtacaccccggtcagcaggaagccatcgaccttcaacctctttgtgttcagcccagacacaggtgctgtctctggctcctaccgagttcgagccctggactactgggcccgaccaggccccttctcggaccctgtgccgtacctggaggtccctgtgccaagagggcccccatccccgggcaatccataagcggccgc

SEQ ID NO: 29 - DNA, 53 bp, Artificial Sequence
  Primer IRES5', synthetic sequence
caactcgagcggccgccccccccccctctccctcccccccccctaacgttact

SEQ ID NO: 30 - DNA, 22 bp, Artificial Sequence
  Primer IRES3', synthetic sequence
caagaagcttccagaggaactg

SEQ ID NO: 31 - DNA, 30 bp, Artificial Sequence
  Primer mPGKP5', synthetic sequence
gcgagatcttaccgggtaggggaggcgctt

SEQ ID NO: 32 - DNA, 30 bp, Artificial Sequence
  Primer mPGKP3', synthetic sequence
gaggaattcgatgatcggtcgaaaggcccg

SEQ ID NO: 33 - DNA, 36 bp, Artificial Sequence
  Primer GS5', synthetic sequence
aatatggccacaaccatggcgacctcagcaagttcc

SEQ ID NO: 34 - DNA, 38 bp, Artificial Sequence
  Primer GS3', synthetic sequence
ggaggatccctcgagttagtttttgtattggaagggct

SEQ ID NO: 35 - DNA, 28 bp, Artificial Sequence
  Primer puro5', synthetic sequence
gcttaagatgaccgagtacaagcccacg

SEQ ID NO: 36 - DNA, 30 bp, Artificial Sequence
  Primer puro3', synthetic sequence
cccatcgtgatggtcaggcaccgggcttgc

SEQ ID NO: 37 - DNA, 44 bp, Artificial Sequence
  Primer SV40polyA5', synthetic sequence
caacaagcggccgccctcgagttccctttagtgagggttaatgc

SEQ ID NO: 38 - DNA, 24 bp, Artificial Sequence
  Primer SV40polyA3', synthetic sequence
cccctgaacctgaaacataaaatg

SEQ ID NO: 39 - DNA, 25 bp, Artificial Sequence
  Primer mIRES-GS5', synthetic sequence
acacgatgataagcttgccacaacc

SEQ ID NO: 40 - DNA, 21 bp, Artificial Sequence
  Primer mIRES-GS3', synthetic sequence
ctccacgatatccctgccata

SEQ ID NO: 41 - DNA, 2076 bp, Artificial Sequence
  CMVE-EF-1 alpha p-IFN beta MAR, synthetic sequence
aagcttaaattatctctaaggcatgtgaactggctgtcttggttttcatctgtacttcatctgctacctctgtgacctgaaacatatttataattccattaagctgtgcatatgatagatttatcatatgtattttccttaaaggatttttgtaagaactaattgaattgatacctgtaaagtctttatcacactacccaataaataataaatctctttgttcagctctctgtttctataaatatgtaccagttttattgtttttagtggtagtgattttattctctttctatatatatacacacacatgtgtgcattcataaatatatacaatttttatgaataaaaaattattagcaatcaatattgaaaaccactgatttttgtttatgtgagcaaacagcagattaaaagaaattcctgcaggagtcaatgggaaaaacccattggagccaagtacactgactcaatagggactttccattgggttttgcccagtacataaggtcaatagggggtgagtcaacaggaaagtcccattggagccaagtacattgagtcaatagggactttccaatgggttttgcccagtacataaggtcaatgggaggtaagccaatgggtttttcccattactgacatgtatactgagtcattagggactttccaatgggttttgcccagtacataaggtcaataggggtgaatcaacaggaaagtcccattggagccaagtacactgagtcaatagggactttccattgggttttgcccagtacaaaaggtcaatagggggtgagtcaatgggtttttcccattattggcacatacataaggtcaataggggtgactagtggagaagagcatgcttgagggctgagtgcccctcagtgggcagagagcacatggcccacagtccctgagaagttggggggaggggtgggcaattgaactggtgcctagagaaggtggggcttgggtaaactgggaaagtgatgtggtgtactggctccacctttttccccagggtgggggagaaccatatataagtgcagtagtctctgtgaacattcaaggttctgccttctccctcctgtgagtttggtaagtcactgactgtctatgcctgggaaagggtgggcaggaggtggggcagtgcaggaaaagtggcactgtgaaccctgcagccctagacaattgtactaaccttcttctctttcctctcctgacaggttggtgtacagtagcttccaacgcgtataatggatccagtcaatatgttcaccccaaaaaagctgtttgttaacttgccaacctcattctaaaatgtatatagaagcccaaaagacaataacaaaaatattcttgtagaacaaaatgggaaagaatgttccactaaatatcaagatttagagcaaagcatgagatgtgtggggatagacagtgaggctgataaaatagagtagagctcagaaacagacccattgatatatgtaagtgacctatgaaaaaaatatggcattttacaatgggaaaatgatggtctttttcttttttagaaaaacagggaaatatatttatatgtaaaaaataaaagggaacccatatgtcataccatacacacaaaaaaattccagtgaattataagtctaaatggagaaggcaaaactttaaatcttttagaaaataatatagaagcatgccatcaagacttcagtgtagagaaaaatttcttatcactcaaagtcctaaccacaaagaaaagattgttaattagattgcatgaatattaagacttatttttaaaattaaaaaaccattaagaaaagtcaggccatagaatgacagaaaatatttgcaacaccccagtaaagagaattgtaatatgcagattataaaaagaagtcttacaaatcagtaaaaaataaaactagacaaaaatttgaacagatgaaagagaaactctaaataatcattacacatgagaaactcaatctcagaaatcagagaactatcattgcatatacactaaattagagaaatattaaaaggctaagtaacatctgtggcgaattc

SEQ ID NO: 42 - DNA, 2130 bp, Artificial Sequence
  IRES-HygroR-mPGKpA, synthetic sequence
acgcgtggtacctctagagtcgacccgggcggccgccccccccccctctccctcccccccccctaacgttactggccgaagccgcttggaataaggccggtgtgcgtttgtctatatgttattttccaccatattgccgtcttttggcaatgtgagggcccggaaacctggccctgtcttcttgacgagcattcctaggggtctttcccctctcgccaaaggaatgcaaggtctgttgaatgtcgtgaaggaagcagttcctctggaagcttcttgaagacaaacaacgtctgtagcgaccctttgcaggcagcggaaccccccacctggcgacaggtgcctctgcggccaaaagccacgtgtataagatacacctgcaaaggcggcacaaccccagtgccacgttgtgagttggatagttgtggaaagagtcaaatggctctcctcaagcgtattcaacaaggggctgaaggatgcccagaaggtaccccattgtatgggatctgatctggggcctcggtgcacatgctttacatgtgtttagtcgaggttaaaaaaacgtctaggccccccgaaccacggggacgtggttttcctttgaaaaacacgatgataatatggccacaaccatgaaaaagcctgaactcaccgcgacgtctgtcgagaagtttctgatcgaaaagttcgacagcgtctccgacctgatgcagctctcggagggcgaagaatctcgtgctttcagcttcgatgtaggagggcgtggatatgtcctgcgggtaaatagctgcgccgatggtttctacaaagatcgttatgttcatcggcactttgcatcggccgcgctcccgattccggaagtgcttgacattggggaattcagcgagagcctgacctattgcatctcccgccgtgcacagggtgtcacgttgcaagacctgcctgaaaccgaactgcccgctgttctgcagccggtcgcggaggccatggatgcgatcgctgcggccgatcttagccagacgagcgggttcggcccattcggaccgcaaggaatcggtcaatacactacgtggcgtgatttcatatgcgcgattgctgatccccatgtgtatcactggcaaactgtgatggacgacaccgtcagtgcgtccgtcgcgcaggctctcgatgagctgatgctttgggccgaggactgccccgaagtccggcacctcgtgcacgcggatttcggctccaacaatgtcctgacggacaatggccgcataacagcggtcattgactggagcgaggcgatgttcggggattcccaatacgaggtcgccaacatcttcttctggaggccgtggttggcttgtatggagcagcagacgcgctacttcgagcggaggcatccggagcttgcaggatcgccgcggctccgggcgtatatgctccgcattggtcttgaccaactctatcagagcttggttgacggcaatttcgatgatgcagcttgggcgcagggtcgatgcgacgcaatcgtccgatccggagccgggactgtcgggcgtacacaaatcgcccgcagaagcgcggccgtctggaccgatggctgtgtagaagtactcgccgatagtggaaaccgacgccccagcactcgtccgagggcaaaggaatagtcgagaaattgatgatctattaagcaataaagacgtccactaaaatggaagtttttcctgtcatactttgttaagaagggtgagaacagagtacctacattttgaatggaaggattggagctacgggggtgggggtggggtgggattagataaatgcctgctctttactgaaggctctttactattgctttatgataatgtttcatagttggatatcataatttaaacaagcaaaaccaaattaagggccagctcattcctccactcacgatctatagatccactagcttggcgtaatcatggtcatagctgtttcctgtgtgaaattgttatccgctcacaattccacacaacatacgagccggaagcataaagtgtaaagcctggggtgcctaatgagtgagctaactcacattaattgcgttgcgctcactgcccgctttccagtcgggaaacctgtcgtgccagcggatcc